European Patent Specification EP 3 334 273 B1, published February 12, 2025. Title: RESISTANCE TO AUSTRALIAN VARIANT OF A. CANDIDA RACE 9 IN BROCCOLI. Applicant: VILMORIN & CIE. The sequence listing filed with the application follows.

SEQUENCE LISTING (42 sequences)

SEQ ID NO: 1 - DNA, 150 bp, Brassica oleracea
  polymorphism (75)..(75): susceptible = T; resistant = C
atttgattgtgtgcctttcccagtttattgaatacaacattgtttcatgaagcaggttgcaggattgcttggtgygagttctgatctttcagcttactgtcctggtccaagtccttcttcagctgatactgaaatcaaacctgatctgca

SEQ ID NO: 2 - DNA, 150 bp, Brassica oleracea
  polymorphism (75)..(75): susceptible = A; resistant = G
agctcttgtctctgaaagaacgtcaaaccttcaaaaaatggcattgaagtttaatcctttggtatctcagccatrcaaactcgcttcctcggctcgtccgccaatctctactttcagatctcccaagttcctctgcctcgcttcttcttc

SEQ ID NO: 3 - DNA, 150 bp, Brassica oleracea
  polymorphism (75)..(75): susceptible = C; resistant = A
ttcaatataagctgcagaaaacaagaggtggtaggtaatagaaaaaaaacctgctcaatgatctcatgtctctgmaggtttcttgaaaaccctcctttcccagtagcacaaaacgagcaacgcagtggacatccaacctaaatcagagag

SEQ ID NO: 4 - DNA, 150 bp, Brassica oleracea
  polymorphism (75)..(75): susceptible = C; resistant = T
tacgagtttggattttaactttttataaaaaagtataattaaaaaatgagcttgaaggacgccagcaaggaatgygggtgatgaatgatgatcgtatcttccgtaagatacggaacacataacgccatctatcttcagacaaagacattc

SEQ ID NO: 5 - DNA, 150 bp, Brassica oleracea
  polymorphism (75)..(75): susceptible = A; resistant = G
cccatgaagttgaggtatccttctccacctagtcccatcgtaatgagccgtatcattttgtgtaaggcgatcccrcggtctacacgtggtgtggcctgtttgtccaccgccatgaaatcatacatgtcctacaaaacagtaagatgttag

SEQ ID NO: 6 - DNA, 151 bp, Brassica oleracea
  polymorphism (76)..(76): susceptible = A; resistant = C
ttaatgttgatgaagaactagaagccatgggtaagaaaatggtcacatattgtggaggactcccattagccgttamagtgctgggaggcttgttagctaataaaaccatggttgaagagtggaaaagaatatatgacgatattcaaactca

SEQ ID NO: 7 - DNA, 151 bp, Brassica oleracea
  polymorphism (76)..(76): susceptible = T; resistant = G
ggactcccattagccgttaaagtgctgggaggcttgttagctaataaaaccatggttgaagagtggaaaagaatakatgacgatattcaaactcagatagttcgcatagatgaaaacagtcaagattcggtttaccgagtattgtctctaa

SEQ ID NO: 8 - DNA, 151 bp, Brassica oleracea
  polymorphism (76)..(76): susceptible = G; resistant = A
ccattagccgttaaagtgctgggaggcttgttagctaataaaaccatggttgaagagtggaaaagaatatatgacratattcaaactcagatagttcgcatagatgaaaacagtcaagattcggtttaccgagtattgtctctaagctatg

SEQ ID NO: 9 - DNA, 151 bp, Brassica oleracea
  polymorphism (76)..(76): susceptible = A; resistant = C
agctaataaaaccatggttgaagagtggaaaagaatatatgacgatattcaaactcagatagttcgcatagatgamaacagtcaagattcggtttaccgagtattgtctctaagctatgaagatttgccaatgcagttaaagcattgcttc

SEQ ID NO: 10 - DNA, 151 bp, Brassica oleracea
  polymorphism (76)..(76): susceptible = G; resistant = A
accatggttgaagagtggaaaagaatatatgacgatattcaaactcagatagttcgcatagatgaaaacagtcaarattcggtttaccgagtattgtctctaagctatgaagatttgccaatgcagttaaagcattgcttcctctacctag

SEQ ID NO: 11 - DNA, 151 bp, Brassica oleracea
  polymorphism (76)..(76): susceptible = T; resistant = G
catggttgaagagtggaaaagaatatatgacgatattcaaactcagatagttcgcatagatgaaaacagtcaagaktcggtttaccgagtattgtctctaagctatgaagatttgccaatgcagttaaagcattgcttcctctacctagct

SEQ ID NO: 12 - DNA, 151 bp, Brassica oleracea
  polymorphism (76)..(76): susceptible = T; resistant = C
ttgtctctaagctatgaagatttgccaatgcagttaaagcattgcttcctctacctagctcattttcccgaagatyacaagatacaagtggagagattgtattatctctgggaagcagaaggaataataacgtcaagtggcgatggagaaa

SEQ ID NO: 13 - DNA, 151 bp, Brassica oleracea
  polymorphism (76)..(76): susceptible = T; resistant = C
atgaagatttgccaatgcagttaaagcattgcttcctctacctagctcattttcccgaagattacaagatacaagyggagagattgtattatctctgggaagcagaaggaataataacgtcaagtggcgatggagaaaccactaggaaaat

SEQ ID NO: 14 - DNA, 150 bp, Brassica oleracea
  polymorphism (75)..(75): susceptible = C; resistant = T
aacttgtctttgatttatttatgttcgctttttcttttgatactacaaaagctaatcatttccaaatctcgaaaygaaagtctagcatatgtacaactcttatgcatctttggcaaaaaaaatgattctcggaaaattacatgttcgtat

SEQ ID NO: 15 - DNA, 150 bp, Brassica oleracea
  polymorphism (75)..(75): susceptible = A; resistant = G
cgatacagttgtatgtacaggctaaaaaaatgtttttttaaagaaaaacataaaactatataacttgttccatartgaatacatacatagtcacgtagatcattcggatttggcaactcttcttatcatgcgcataatcaaacctccaaa

SEQ ID NO: 16 - DNA, 150 bp, Brassica oleracea
  polymorphism (75)..(75): susceptible = T; resistant = G
taattgatcagaatcttcacatcttttaagagaaaccaaaaaatggtctacacaccatcctcttttgcttactakcatgcatgataagtagaaacaaaagaaaagaagaagcatctctatgtttacaaagtggcagcaaccaaatcagga

SEQ ID NO: 17 - DNA, 150 bp, Brassica oleracea
  polymorphism (75)..(75): susceptible = G; resistant = A
atggaggatacaccttccgtgtccggagataaggtgagagctttacgcgcgtgattcagagctgagatcaagtcrccgctgttgaatttcgattccgctagggtgtattgcctcgttaccagtgtctcggtctgatcctgaagctgccat

SEQ ID NO: 18 - DNA, 150 bp, Brassica oleracea
  polymorphism (75)..(75): susceptible = A; resistant = C
ttcgtgagctgattcttggtggggtatgttgatttgccagataacaatgaaagtcataagaagcaagaacgtccmgattcccaaactccaccaccggttccttcaggaccatgttctgaatctatagatacaagctccgtctactcagaa

SEQ ID NO: 19 - DNA, 150 bp, Brassica oleracea
  polymorphism (75)..(75): susceptible = T; resistant = G
ttctttttatccgccttctcaatttgccgatttagggtttctcttttggttgatttgtcggcgtcactgttgttktttttattccgtacagtttctggagaagttcccgaggtgcctgtggtttcaacgaagtcaggtttgctcttcgag

SEQ ID NO: 20 - DNA, 150 bp, Brassica oleracea
  polymorphism (75)..(75): susceptible = A; resistant = G
aataactgtaacatttaagactcttcttgctataataacttatgttttctgttccagcttgttgacccaaagacrggagatgagaaacccattacagtctctgttgatgatgggatccgaccaagcacaacccttgctactcttgggaag

SEQ ID NO: 21 - DNA, 150 bp, Brassica oleracea
  polymorphism (75)..(75): susceptible = T; resistant = C
acgaatctcgtgatggtcatcaaatccgtacggtaagcatctgcttcgtgatccatctttgtttctcgctctccycgttatgaagcggatacctttttaatcagatgtttagaagatattatatataacctgcattatttttctttttaa

SEQ ID NO: 22 - DNA, 150 bp, Brassica oleracea
  polymorphism (75)..(75): susceptible = G; resistant = C
aacctcttgggatggattcttttgggagtgtttggtttgatctggactttctactttacctacacttcttctctsgacgaggatgaagaatctggtctttcactctaaacatgaactgtatatgttcttcatcagtgtcatctctctcct

SEQ ID NO: 23 - DNA, 150 bp, Brassica oleracea
  polymorphism (75)..(75): susceptible = T; resistant = C
aaaatagaaaaaattgaatagttggtattcaaacattgattctaagcttgccaaattgatccggatcactagttytactggttttagtcggtaaaaccggatattttctttaaatcaatttttaaaccaaactgaactcggcttattcaa

SEQ ID NO: 24 - DNA, 150 bp, Brassica oleracea
  polymorphism (75)..(75): susceptible = G; resistant = A
tccgttatgatacttcaatcgcctttattggcatcggaacaaagaaactctctgccgacgaggagcaaacacgcrgagaggagaaaagtaggagaggtagctggaggagcggcggccgagtgtgcggcggtctggtgttgctgtccttgc

SEQ ID NO: 25 - DNA, 150 bp, Brassica oleracea
  polymorphism (75)..(75): susceptible = A; resistant = G
atttcgagcaactcgcgaagaagctggaagaggcttctccacttgaaatcatggacaaagctctccagaaattcrgaagcaacatcgcaattgctttcaggtaatcaatcgattcaattaaagatccaaaagaatagaaagaacttgaat

SEQ ID NO: 26 - DNA, 150 bp, Brassica oleracea
  polymorphism (75)..(75): susceptible = T; resistant = C
tatagttccgtcttaagtttgtttacatgtacaatatgcttttacgatttcagtccttggcttgaggcaccctayaaagatgccgcagagaaaacaccgggcggaaagttgacaatcaatgggtttctgtctgaggtttgtatgcttgct

SEQ ID NO: 27 - DNA, 150 bp, Brassica oleracea
  polymorphism (75)..(75): susceptible = C; resistant = G
attgtttctcttcgtagctgccaccgcaacggcagccgctacaccaaccaaacgcgcaaactaccttttcacacsgcacgcaaaagcagtcgcgggaatatgcactgtaatccaaacaaacacaagtctatgctgcaaaacccttaaaca

SEQ ID NO: 28 - DNA, 150 bp, Brassica oleracea
  polymorphism (75)..(75): susceptible = G; resistant = C
tgcaaatggcaggcacactatatcagcggcacaagcagcctttcttgatgatcacttgggatctatatctccagsgaagcttgcggattttgttgtattgtcaacaaattcatgggacgagttctcaaaagacggttctgcttcggtttt

SEQ ID NO: 29 - DNA, 150 bp, Brassica oleracea
  polymorphism (75)..(75): susceptible = A; resistant = G
ctagatttatgtaatttgaagggttcaaatgtgactggtggggttggcccttttggtctgatcaccttggctacrtctgacctacaagaatacactcccgtcttcttcagagtcttcaaagatggcacaaccaacaagcctaaggtcctc

SEQ ID NO: 30 - DNA, 150 bp, Brassica oleracea
  polymorphism (75)..(75): susceptible = C; resistant = T
gagtaagttaaaatctaaagacaagggcaagtcttcaaaaaagaaggaagcaacgagtaatgcaaaagaaggacygaggacacctggaggcgaagaagcgctttcaaatgtaaccaaggagaaggctgctgctgccaaactatatattga

SEQ ID NO: 31 - DNA, 150 bp, Brassica oleracea
  polymorphism (75)..(75): susceptible = C; resistant = T
gctgtcccagatatctggagatcttctgcagaaaagtatggggataaaattgcacttgtagatccttaccatgayccacctttgaaattgacatacaaccaggtatatgtctattgtcgctgtagacttggtgagcgagcaacggagttc

SEQ ID NO: 32 - DNA, 150 bp, Brassica oleracea
  polymorphism (75)..(75): susceptible = G; resistant = A
cgaaacctccagcagattccagaaaggttgaaacttcctcaaagcccgagaccaagaagaagcgatctagtgagrcagatgaaggcgaagaagcaaagagggtcaagagggtttcaggggaagacgaccacaaaaagagtaagggagagg

SEQ ID NO: 33 - DNA, 150 bp, Brassica oleracea
  polymorphism (75)..(75): susceptible = G; resistant = T
atttcaattcgtgttattggaatcataccttttttttctttccaggtgatgttatttgccggttcggaaacaacktcagtgacattagagtgggctatgtctaaccttctaaatcatccagatgttctagcgaaagtaaagacggaacta

SEQ ID NO: 34 - DNA, 150 bp, Brassica oleracea
  polymorphism (75)..(75): susceptible = A; resistant = G
gattttcagtttacacatcccatcaatcacaattatatttattaaaaaaaaaagtgctaacttacaatcttatcraagagttctcctcctgtaacatactccaagatgataaatatttttgtcttgcttgccatcacctgcaaaatcaca

SEQ ID NO: 35 - DNA, 150 bp, Brassica oleracea
  polymorphism (75)..(75): susceptible =G; resistant = A
agttttagatacaaagaagtgtctctctgcaatgaaagaaccgatttaagaaaagtaccagcggttgtggtgccrtcctttttaaacacaggcttcagcttcccaagagtagcaagggttgtgcttggtcggatcccatcatcaacagaa

SEQ ID NO: 36 - DNA, 150 bp, Brassica oleracea
  polymorphism (75)..(75): susceptible = A; resistant = G
ctcacttgttattttccacatcttttgttcactgagattagtcccttttggcagaattggtattgtgcatcaaaracacaagcagaaagtgaagctttcgaatttgcaaaacgaaccgggattagtctcgtcagcatttgccctaccatg

SEQ ID NO: 37 - DNA, 150 bp, Brassica oleracea
  polymorphism (75)..(75): susceptible = A; resistant = C
taaaacccaaagccatataccacttcaacattatattattttttacgttattggatttaaaagtcaacgacctcmaagttccatcaaccaatctttgtcggaatactctgttcatgcctgaaaaagttctcaggatcaaactcaccttta

SEQ ID NO: 38 - DNA, 150 bp, Brassica oleracea
  polymorphism (75)..(75): susceptible = C; resistant = G
caatcaagataatcctctgcatcttcataatcagtgaggacagacaccgtgcattgcagaaacggcagttctttsggttggattggtgggaacctacgatccctcagggcactgtgatattgacataaatcaaaaaggtacatttataac

SEQ ID NO: 39 - DNA, 150 bp, Brassica oleracea
  polymorphism (75)..(75): susceptible = A; resistant = G
ggcggcctcccttcaacccgcatgcttggacctccacttcgccgggaaacatcctccgcctctcaaacacaccarcgccaccttcctccgctgcgtctcctctccgaatttccccgagcctgactcgcctgacgccaatctcaccaaaga

SEQ ID NO: 40 - DNA, 150 bp, Brassica oleracea
  polymorphism (75)..(75): susceptible = A; resistant = G
agcgttggaagagcatctttctgatacttgtttccaagctcagagatctttcccagccacaagttgttccaagcraatataacagcgatcacagatggaccgaggatcacttggttaagcagaacctaacaaagggatcgataagataca

SEQ ID NO: 41 - DNA, 20 bp, Brassica oleracea
cgctcaaacggttaacatga

SEQ ID NO: 42 - DNA, 20 bp, Brassica oleracea
ccatcgccacttgacgttat